European Patent Specification EP 3 722 442 B1, published April 5, 2023. Title: DE NOVO SYNTHESIZED GENE LIBRARIES. Applicant: TWIST BIOSCIENCE CORPORATION. The sequence listing filed with the application follows.

SEQUENCE LISTING (81 sequences)

SEQ ID NO: 1 - DNA, 62 bp, Artificial Sequence
  Description of Artificial Sequence: Synthetic oligonucleotide
  modified_base (51)..(52): Thymidine-succinyl hexamide CED phosphoramidite
agacaatcaaccatttggggtggacagccttgacctctagacttcggcattttttttttttt

SEQ ID NO: 2 - DNA, 112 bp, Artificial Sequence
  Description of Artificial Sequence: Synthetic polynucleotide
  modified_base (101)..(102): Thymidine-succinyl hexamide CED phosphoramidite
cgggatccttatcgtcatcgtcgtacagatcccgacccatttgctgtccaccagtcatgctagccataccatgatgatgatgatgatgagaaccccgcattttttttttttt

SEQ ID NO: 3 - DNA, 19 bp, Artificial Sequence
  Description of Artificial Sequence: Synthetic oligonucleotide
atgcggggttctcatcatc

SEQ ID NO: 4 - DNA, 20 bp, Artificial Sequence
  Description of Artificial Sequence: Synthetic oligonucleotide
cgggatccttatcgtcatcg

SEQ ID NO: 5 - DNA, 19 bp, Artificial Sequence
  Description of Artificial Sequence: Synthetic oligonucleotide
atgcggggttctcatcatc

SEQ ID NO: 6 - DNA, 20 bp, Artificial Sequence
  Description of Artificial Sequence: Synthetic oligonucleotide
cgggatccttatcgtcatcg

SEQ ID NO: 7 - DNA, 62 bp, Artificial Sequence
  Description of Artificial Sequence: Synthetic oligonucleotide
atgaccatgattacggattcactggccgtcgttttacaacgtcgtgactgggaaaaccctgg

SEQ ID NO: 8 - DNA, 72 bp, Artificial Sequence
  Description of Artificial Sequence: Synthetic oligonucleotide
gccagctggcgaaagggggatgtgctgcaaggcgattaagttgggtaacgccagggttttcccagtcacgac

SEQ ID NO: 9 - DNA, 70 bp, Artificial Sequence
  Description of Artificial Sequence: Synthetic oligonucleotide
ccccctttcgccagctggcgtaatagcgaagaggcccgcaccgatcgcccttcccaacagttgcgcagcc

SEQ ID NO: 10 - DNA, 69 bp, Artificial Sequence
  Description of Artificial Sequence: Synthetic oligonucleotide
cggcaccgcttctggtgccggaaaccaggcaaagcgccattcgccattcaggctgcgcaactgttggga

SEQ ID NO: 11 - DNA, 70 bp, Artificial Sequence
  Description of Artificial Sequence: Synthetic oligonucleotide
caccagaagcggtgccggaaagctggctggagtgcgatcttcctgaggccgatactgtcgtcgtcccctc

SEQ ID NO: 12 - DNA, 75 bp, Artificial Sequence
  Description of Artificial Sequence: Synthetic oligonucleotide
gataggtcacgttggtgtagatgggcgcatcgtaaccgtgcatctgccagtttgaggggacgacgacagtatcgg

SEQ ID NO: 13 - DNA, 74 bp, Artificial Sequence
  Description of Artificial Sequence: Synthetic oligonucleotide
cccatctacaccaacgtgacctatcccattacggtcaatccgccgtttgttcccacggagaatccgacgggttg

SEQ ID NO: 14 - DNA, 72 bp, Artificial Sequence
  Description of Artificial Sequence: Synthetic oligonucleotide
gtctggccttcctgtagccagctttcatcaacattaaatgtgagcgagtaacaacccgtcggattctccgtg

SEQ ID NO: 15 - DNA, 73 bp, Artificial Sequence
  Description of Artificial Sequence: Synthetic oligonucleotide
gctggctacaggaaggccagacgcgaattatttttgatggcgttaactcggcgtttcatctgtggtgcaacgg

SEQ ID NO: 16 - DNA, 74 bp, Artificial Sequence
  Description of Artificial Sequence: Synthetic oligonucleotide
caggtcaaattcagacggcaaacgactgtcctggccgtaaccgacccagcgcccgttgcaccacagatgaaacg

SEQ ID NO: 17 - DNA, 72 bp, Artificial Sequence
  Description of Artificial Sequence: Synthetic oligonucleotide
cgtttgccgtctgaatttgacctgagcgcatttttacgcgccggagaaaaccgcctcgcggtgatggtgctg

SEQ ID NO: 18 - DNA, 72 bp, Artificial Sequence
  Description of Artificial Sequence: Synthetic oligonucleotide
gccgctcatccgccacatatcctgatcttccagataactgccgtcactccagcgcagcaccatcaccgcgag

SEQ ID NO: 19 - DNA, 77 bp, Artificial Sequence
  Description of Artificial Sequence: Synthetic oligonucleotide
aggatatgtggcggatgagcggcattttccgtgacgtctcgttgctgcataaaccgactacacaaatcagcgatttc

SEQ ID NO: 20 - DNA, 78 bp, Artificial Sequence
  Description of Artificial Sequence: Synthetic oligonucleotide
ctccagtacagcgcggctgaaatcatcattaaagcgagtggcaacatggaaatcgctgatttgtgtagtcggtttatg

SEQ ID NO: 21 - DNA, 75 bp, Artificial Sequence
  Description of Artificial Sequence: Synthetic oligonucleotide
atttcagccgcgctgtactggaggctgaagttcagatgtgcggcgagttgcgtgactacctacgggtaacagttt

SEQ ID NO: 22 - DNA, 71 bp, Artificial Sequence
  Description of Artificial Sequence: Synthetic oligonucleotide
aaaggcgcggtgccgctggcgacctgcgtttcaccctgccataaagaaactgttacccgtaggtagtcacg

SEQ ID NO: 23 - DNA, 70 bp, Artificial Sequence
  Description of Artificial Sequence: Synthetic oligonucleotide
gcggcaccgcgcctttcggcggtgaaattatcgatgagcgtggtggttatgccgatcgcgtcacactacg

SEQ ID NO: 24 - DNA, 74 bp, Artificial Sequence
  Description of Artificial Sequence: Synthetic oligonucleotide
gatagagattcgggatttcggcgctccacagtttcgggttttcgacgttcagacgtagtgtgacgcgatcggca

SEQ ID NO: 25 - DNA, 74 bp, Artificial Sequence
  Description of Artificial Sequence: Synthetic oligonucleotide
gagcgccgaaatcccgaatctctatcgtgcggtggttgaactgcacaccgccgacggcacgctgattgaagcag

SEQ ID NO: 26 - DNA, 73 bp, Artificial Sequence
  Description of Artificial Sequence: Synthetic oligonucleotide
cagcagcagaccattttcaatccgcacctcgcggaaaccgacatcgcaggcttctgcttcaatcagcgtgccg

SEQ ID NO: 27 - DNA, 74 bp, Artificial Sequence
  Description of Artificial Sequence: Synthetic oligonucleotide
cggattgaaaatggtctgctgctgctgaacggcaagccgttgctgattcgaggcgttaaccgtcacgagcatca

SEQ ID NO: 28 - DNA, 75 bp, Artificial Sequence
  Description of Artificial Sequence: Synthetic oligonucleotide
gcaggatatcctgcaccatcgtctgctcatccatgacctgaccatgcagaggatgatgctcgtgacggttaacgc

SEQ ID NO: 29 - DNA, 75 bp, Artificial Sequence
  Description of Artificial Sequence: Synthetic oligonucleotide
cagacgatggtgcaggatatcctgctgatgaagcagaacaactttaacgccgtgcgctgttcgcattatccgaac

SEQ ID NO: 30 - DNA, 74 bp, Artificial Sequence
  Description of Artificial Sequence: Synthetic oligonucleotide
tccaccacatacaggccgtagcggtcgcacagcgtgtaccacagcggatggttcggataatgcgaacagcgcac

SEQ ID NO: 31 - DNA, 75 bp, Artificial Sequence
  Description of Artificial Sequence: Synthetic oligonucleotide
gctacggcctgtatgtggtggatgaagccaatattgaaacccacggcatggtgccaatgaatcgtctgaccgatg

SEQ ID NO: 32 - DNA, 73 bp, Artificial Sequence
  Description of Artificial Sequence: Synthetic oligonucleotide
gcaccattcgcgttacgcgttcgctcatcgccggtagccagcgcggatcatcggtcagacgattcattggcac

SEQ ID NO: 33 - DNA, 73 bp, Artificial Sequence
  Description of Artificial Sequence: Synthetic oligonucleotide
cgcgtaacgcgaatggtgcagcgcgatcgtaatcacccgagtgtgatcatctggtcgctggggaatgaatcag

SEQ ID NO: 34 - DNA, 78 bp, Artificial Sequence
  Description of Artificial Sequence: Synthetic oligonucleotide
ggatcgacagatttgatccagcgatacagcgcgtcgtgattagcgccgtggcctgattcattccccagcgaccagatg

SEQ ID NO: 35 - DNA, 72 bp, Artificial Sequence
  Description of Artificial Sequence: Synthetic oligonucleotide
gtatcgctggatcaaatctgtcgatccttcccgcccggtgcagtatgaaggcggcggagccgacaccacggc

SEQ ID NO: 36 - DNA, 71 bp, Artificial Sequence
  Description of Artificial Sequence: Synthetic oligonucleotide
cgggaagggctggtcttcatccacgcgcgcgtacatcgggcaaataatatcggtggccgtggtgtcggctc

SEQ ID NO: 37 - DNA, 73 bp, Artificial Sequence
  Description of Artificial Sequence: Synthetic oligonucleotide
tggatgaagaccagcccttcccggctgtgccgaaatggtccatcaaaaaatggctttcgctacctggagagac

SEQ ID NO: 38 - DNA, 73 bp, Artificial Sequence
  Description of Artificial Sequence: Synthetic oligonucleotide
ccaagactgttacccatcgcgtgggcgtattcgcaaaggatcagcgggcgcgtctctccaggtagcgaaagcc

SEQ ID NO: 39 - DNA, 73 bp, Artificial Sequence
  Description of Artificial Sequence: Synthetic oligonucleotide
cgcgatgggtaacagtcttggcggtttcgctaaatactggcaggcgtttcgtcagtatccccgtttacagggc

SEQ ID NO: 40 - DNA, 78 bp, Artificial Sequence
  Description of Artificial Sequence: Synthetic oligonucleotide
gccgttttcatcatatttaatcagcgactgatccacccagtcccagacgaagccgccctgtaaacggggatactgacg

SEQ ID NO: 41 - DNA, 76 bp, Artificial Sequence
  Description of Artificial Sequence: Synthetic oligonucleotide
cagtcgctgattaaatatgatgaaaacggcaacccgtggtcggcttacggcggtgattttggcgatacgccgaacg

SEQ ID NO: 42 - DNA, 67 bp, Artificial Sequence
  Description of Artificial Sequence: Synthetic oligonucleotide
gcggcgtgcggtcggcaaagaccagaccgttcatacagaactggcgatcgttcggcgtatcgccaaa

SEQ ID NO: 43 - DNA, 71 bp, Artificial Sequence
  Description of Artificial Sequence: Synthetic oligonucleotide
cgaccgcacgccgcatccagcgctgacggaagcaaaacaccagcagcagtttttccagttccgtttatccg

SEQ ID NO: 44 - DNA, 79 bp, Artificial Sequence
  Description of Artificial Sequence: Synthetic oligonucleotide
ctcgttatcgctatgacggaacaggtattcgctggtcacttcgatggtttgcccggataaacggaactggaaaaactgc

SEQ ID NO: 45 - DNA, 75 bp, Artificial Sequence
  Description of Artificial Sequence: Synthetic oligonucleotide
aatacctgttccgtcatagcgataacgagctcctgcactggatggtggcgctggatggtaagccgctggcaagcg

SEQ ID NO: 46 - DNA, 76 bp, Artificial Sequence
  Description of Artificial Sequence: Synthetic oligonucleotide
gttcaggcagttcaatcaactgtttaccttgtggagcgacatccagaggcacttcaccgcttgccagcggcttacc

SEQ ID NO: 47 - DNA, 78 bp, Artificial Sequence
  Description of Artificial Sequence: Synthetic oligonucleotide
caaggtaaacagttgattgaactgcctgaactaccgcagccggagagcgccgggcaactctggctcacagtacgcgta

SEQ ID NO: 48 - DNA, 71 bp, Artificial Sequence
  Description of Artificial Sequence: Synthetic oligonucleotide
gcgctgatgtgcccggcttctgaccatgcggtcgcgttcggttgcactacgcgtactgtgagccagagttg

SEQ ID NO: 49 - DNA, 67 bp, Artificial Sequence
  Description of Artificial Sequence: Synthetic oligonucleotide
ccgggcacatcagcgcctggcagcagtggcgtctggcggaaaacctcagtgtgacgctccccgccgc

SEQ ID NO: 50 - DNA, 71 bp, Artificial Sequence
  Description of Artificial Sequence: Synthetic oligonucleotide
ccagctcgatgcaaaaatccatttcgctggtggtcagatgcgggatggcgtgggacgcggcggggagcgtc

SEQ ID NO: 51 - DNA, 78 bp, Artificial Sequence
  Description of Artificial Sequence: Synthetic oligonucleotide
cgaaatggatttttgcatcgagctgggtaataagcgttggcaatttaaccgccagtcaggctttctttcacagatgtg

SEQ ID NO: 52 - DNA, 74 bp, Artificial Sequence
  Description of Artificial Sequence: Synthetic oligonucleotide
tgaactgatcgcgcagcggcgtcagcagttgttttttatcgccaatccacatctgtgaaagaaagcctgactgg

SEQ ID NO: 53 - DNA, 73 bp, Artificial Sequence
  Description of Artificial Sequence: Synthetic oligonucleotide
gccgctgcgcgatcagttcacccgtgcaccgctggataacgacattggcgtaagtgaagcgacccgcattgac

SEQ ID NO: 54 - DNA, 71 bp, Artificial Sequence
  Description of Artificial Sequence: Synthetic oligonucleotide
ggcctggtaatggcccgccgccttccagcgttcgacccaggcgttagggtcaatgcgggtcgcttcactta

SEQ ID NO: 55 - DNA, 70 bp, Artificial Sequence
  Description of Artificial Sequence: Synthetic oligonucleotide
cgggccattaccaggccgaagcagcgttgttgcagtgcacggcagatacacttgctgatgcggtgctgat

SEQ ID NO: 56 - DNA, 75 bp, Artificial Sequence
  Description of Artificial Sequence: Synthetic oligonucleotide
tccggctgataaataaggttttcccctgatgctgccacgcgtgagcggtcgtaatcagcaccgcatcagcaagtg

SEQ ID NO: 57 - DNA, 78 bp, Artificial Sequence
  Description of Artificial Sequence: Synthetic oligonucleotide
ggggaaaaccttatttatcagccggaaaacctaccggattgatggtagtggtcaaatggcgattaccgttgatgttga

SEQ ID NO: 58 - DNA, 75 bp, Artificial Sequence
  Description of Artificial Sequence: Synthetic oligonucleotide
ggcagttcaggccaatccgcgccggatgcggtgtatcgctcgccacttcaacatcaacggtaatcgccatttgac

SEQ ID NO: 59 - DNA, 71 bp, Artificial Sequence
  Description of Artificial Sequence: Synthetic oligonucleotide
gcggattggcctgaactgccagctggcgcaggtagcagagcgggtaaactggctcggattagggccgcaag

SEQ ID NO: 60 - DNA, 72 bp, Artificial Sequence
  Description of Artificial Sequence: Synthetic oligonucleotide
ggcagatcccagcggtcaaaacaggcggcagtaaggcggtcgggatagttttcttgcggccctaatccgagc

SEQ ID NO: 61 - DNA, 72 bp, Artificial Sequence
  Description of Artificial Sequence: Synthetic oligonucleotide
gttttgaccgctgggatctgccattgtcagacatgtataccccgtacgtcttcccgagcgaaaacggtctgc

SEQ ID NO: 62 - DNA, 69 bp, Artificial Sequence
  Description of Artificial Sequence: Synthetic oligonucleotide
gtcgccgcgccactggtgtgggccataattcaattcgcgcgtcccgcagcgcagaccgttttcgctcgg

SEQ ID NO: 63 - DNA, 72 bp, Artificial Sequence
  Description of Artificial Sequence: Synthetic oligonucleotide
accagtggcgcggcgacttccagttcaacatcagccgctacagtcaacagcaactgatggaaaccagccatc

SEQ ID NO: 64 - DNA, 75 bp, Artificial Sequence
  Description of Artificial Sequence: Synthetic oligonucleotide
gaaaccgtcgatattcagccatgtgccttcttccgcgtgcagcagatggcgatggctggtttccatcagttgctg

SEQ ID NO: 65 - DNA, 71 bp, Artificial Sequence
  Description of Artificial Sequence: Synthetic oligonucleotide
catggctgaatatcgacggtttccatatggggattggtggcgacgactcctggagcccgtcagtatcggcg

SEQ ID NO: 66 - DNA, 74 bp, Artificial Sequence
  Description of Artificial Sequence: Synthetic oligonucleotide
ttatttttgacaccagaccaactggtaatggtagcgaccggcgctcagctggaattccgccgatactgacgggc

SEQ ID NO: 67 - DNA, 3075 bp, Artificial Sequence
  Description of Artificial Sequence: Synthetic polynucleotide
atgaccatgattacggattcactggccgtcgttttacaacgtcgtgactgggaaaaccctggcgttacccaacttaatcgccttgcagcacatccccctttcgccagctggcgtaatagcgaagaggcccgcaccgatcgcccttcccaacagttgcgcagcctgaatggcgaatggcgctttgcctggtttccggcaccagaagcggtgccggaaagctggctggagtgcgatcttcctgaggccgatactgtcgtcgtcccctcaaactggcagatgcacggttacgatgcgcccatctacaccaacgtgacctatcccattacggtcaatccgccgtttgttcccacggagaatccgacgggttgttactcgctcacatttaatgttgatgaaagctggctacaggaaggccagacgcgaattatttttgatggcgttaactcggcgtttcatctgtggtgcaacgggcgctgggtcggttacggccaggacagtcgtttgccgtctgaatttgacctgagcgcatttttacgcgccggagaaaaccgcctcgcggtgatggtgctgcgctggagtgacggcagttatctggaagatcaggatatgtggcggatgagcggcattttccgtgacgtctcgttgctgcataaaccgactacacaaatcagcgatttccatgttgccactcgctttaatgatgatttcagccgcgctgtactggaggctgaagttcagatgtgcggcgagttgcgtgactacctacgggtaacagtttctttatggcagggtgaaacgcaggtcgccagcggcaccgcgcctttcggcggtgaaattatcgatgagcgtggtggttatgccgatcgcgtcacactacgtctgaacgtcgaaaacccgaaactgtggagcgccgaaatcccgaatctctatcgtgcggtggttgaactgcacaccgccgacggcacgctgattgaagcagaagcctgcgatgtcggtttccgcgaggtgcggattgaaaatggtctgctgctgctgaacggcaagccgttgctgattcgaggcgttaaccgtcacgagcatcatcctctgcatggtcaggtcatggatgagcagacgatggtgcaggatatcctgctgatgaagcagaacaactttaacgccgtgcgctgttcgcattatccgaaccatccgctgtggtacacgctgtgcgaccgctacggcctgtatgtggtggatgaagccaatattgaaacccacggcatggtgccaatgaatcgtctgaccgatgatccgcgctggctaccggcgatgagcgaacgcgtaacgcgaatggtgcagcgcgatcgtaatcacccgagtgtgatcatctggtcgctggggaatgaatcaggccacggcgctaatcacgacgcgctgtatcgctggatcaaatctgtcgatccttcccgcccggtgcagtatgaaggcggcggagccgacaccacggccaccgatattatttgcccgatgtacgcgcgcgtggatgaagaccagcccttcccggctgtgccgaaatggtccatcaaaaaatggctttcgctacctggagagacgcgcccgctgatcctttgcgaatacgcccacgcgatgggtaacagtcttggcggtttcgctaaatactggcaggcgtttcgtcagtatccccgtttacagggcggcttcgtctgggactgggtggatcagtcgctgattaaatatgatgaaaacggcaacccgtggtcggcttacggcggtgattttggcgatacgccgaacgatcgccagttctgtatgaacggtctggtctttgccgaccgcacgccgcatccagcgctgacggaagcaaaacaccagcagcagtttttccagttccgtttatccgggcaaaccatcgaagtgaccagcgaatacctgttccgtcatagcgataacgagctcctgcactggatggtggcgctggatggtaagccgctggcaagcggtgaagtgcctctggatgtcgctccacaaggtaaacagttgattgaactgcctgaactaccgcagccggagagcgccgggcaactctggctcacagtacgcgtagtgcaaccgaacgcgaccgcatggtcagaagccgggcacatcagcgcctggcagcagtggcgtctggcggaaaacctcagtgtgacgctccccgccgcgtcccacgccatcccgcatctgaccaccagcgaaatggatttttgcatcgagctgggtaataagcgttggcaatttaaccgccagtcaggctttctttcacagatgtggattggcgataaaaaacaactgctgacgccgctgcgcgatcagttcacccgtgcaccgctggataacgacattggcgtaagtgaagcgacccgcattgaccctaacgcctgggtcgaacgctggaaggcggcgggccattaccaggccgaagcagcgttgttgcagtgcacggcagatacacttgctgatgcggtgctgattacgaccgctcacgcgtggcagcatcaggggaaaaccttatttatcagccggaaaacctaccggattgatggtagtggtcaaatggcgattaccgttgatgttgaagtggcgagcgatacaccgcatccggcgcggattggcctgaactgccagctggcgcaggtagcagagcgggtaaactggctcggattagggccgcaagaaaactatcccgaccgccttactgccgcctgttttgaccgctgggatctgccattgtcagacatgtataccccgtacgtcttcccgagcgaaaacggtctgcgctgcgggacgcgcgaattgaattatggcccacaccagtggcgcggcgacttccagttcaacatcagccgctacagtcaacagcaactgatggaaaccagccatcgccatctgctgcacgcggaagaaggcacatggctgaatatcgacggtttccatatggggattggtggcgacgactcctggagcccgtcagtatcggcggaattccagctgagcgccggtcgctaccattaccagttggtctggtgtcaaaaataa

SEQ ID NO: 68 - DNA, 27 bp, Artificial Sequence
  Description of Artificial Sequence: Synthetic oligonucleotide
atgaccatgattacggattcactggcc

SEQ ID NO: 69 - DNA, 31 bp, Artificial Sequence
  Description of Artificial Sequence: Synthetic oligonucleotide
ttatttttgacaccagaccaactggtaatgg

SEQ ID NO: 70 - DNA, 931 bp, Artificial Sequence
  Description of Artificial Sequence: Synthetic polynucleotide
atgaccatgattacggattcactggccgtcgttttacaacgtcgtgactgggaaaaccctggcgttacccaacttaatcgccttgcagcacatccccctttcgccagctggcgtaatagcgaagaggcccgcaccgatcgcccttcccaacagttgcgcagcctgaatggcgaatggcgctttgcctggtttccggcaccagaagcggtgccggaaagctggctggagtgcgatcttcctgaggccgatactgtcgtcgtcccctcaaactggcagatgcacggttacgatgcgcccatctacaccaacgtgacctatcccattacggtcaatccgccgtttgttcccacggagaatccgacgggttgttactcgctcacatttaatgttgatgaaagctggctacaggaaggccagacgcgaattatttttgatggcgttaactcggcgtttcatctgtggtgcaacgggcgctgggtcggttacggccaggacagtcgtttgccgtctgaatttgacctgagcgcatttttacgcgccggagaaaaccgcctcgcggtgatggtgctgcgctggagtgacggcagttatctggaagatcaggatatgtggcggatgagcggcattttccgtgacgtctcgttgctgcataaaccgactacacaaatcagcgatttccatgttgccactcgctttaatgatgatttcagccgcgctgtactggaggctgaagttcagatgtgcggcgagttgcgtgactacctacgggtaacagtttctttatggcagggtgaaacgcaggtcgccagcggcaccgcgcctttcggcggtgaaattatcgatgagcgtggtggttatgccgatcgcgtcacactacgtctgaacgtcgaaaacccgaaactgtggagcgccgaaatcccgaatctctatc

SEQ ID NO: 71 - DNA, 163 bp, Artificial Sequence
  Description of Artificial Sequence: Synthetic polynucleotide
atgaccatgattacggattcactggccgtcgttttacaacgtcgtgactgggaaaaccctggcgttacccaacttaatcgccttgcagcacatccccctttcgccagctggcgtaatagcgaagaggcccgcaccgatcgcccttcccaacagttgcgcagcc

SEQ ID NO: 72 - DNA, 175 bp, Artificial Sequence
  Description of Artificial Sequence: Synthetic polynucleotide
gataggtcacgttggtgtagatgggcgcatcgtaaccgtgcatctgccagtttgaggggacgacgacagtatcggcctcaggaagatcgcactccagccagctttccggcaccgcttctggtgccggaaaccaggcaaagcgccattcgccattcaggctgcgcaactgttggga

SEQ ID NO: 73 - DNA, 176 bp, Artificial Sequence
  Description of Artificial Sequence: Synthetic polynucleotide
cccatctacaccaacgtgacctatcccattacggtcaatccgccgtttgttcccacggagaatccgacgggttgttactcgctcacatttaatgttgatgaaagctggctacaggaaggccagacgcgaattatttttgatggcgttaactcggcgtttcatctgtggtgcaacgg

SEQ ID NO: 74 - DNA, 176 bp, Artificial Sequence
  Description of Artificial Sequence: Synthetic polynucleotide
gccgctcatccgccacatatcctgatcttccagataactgccgtcactccagcgcagcaccatcaccgcgaggcggttttctccggcgcgtaaaaatgcgctcaggtcaaattcagacggcaaacgactgtcctggccgtaaccgacccagcgcccgttgcaccacagatgaaacg

SEQ ID NO: 75 - DNA, 177 bp, Artificial Sequence
  Description of Artificial Sequence: Synthetic polynucleotide
aggatatgtggcggatgagcggcattttccgtgacgtctcgttgctgcataaaccgactacacaaatcagcgatttccatgttgccactcgctttaatgatgatttcagccgcgctgtactggaggctgaagttcagatgtgcggcgagttgcgtgactacctacgggtaacagttt

SEQ ID NO: 76 - DNA, 178 bp, Artificial Sequence
  Description of Artificial Sequence: Synthetic polynucleotide
gatagagattcgggatttcggcgctccacagtttcgggttttcgacgttcagacgtagtgtgacgcgatcggcataaccaccacgctcatcgataatttcaccgccgaaaggcgcggtgccgctggcgacctgcgtttcaccctgccataaagaaactgttacccgtaggtagtcacg

SEQ ID NO: 77 - DNA, 27 bp, Artificial Sequence
  Description of Artificial Sequence: Synthetic oligonucleotide
atgaccatgattacggattcactggcc

SEQ ID NO: 78 - DNA, 27 bp, Artificial Sequence
  Description of Artificial Sequence: Synthetic oligonucleotide
gatagagattcgggatttcggcgctcc

SEQ ID NO: 79 - DNA, 134 bp, Artificial Sequence
  Description of Artificial Sequence: Synthetic polynucleotide
atctttgagtcttctgcttggtcagacgagtgcatgtgcgtgacaaattggcgcgaggagctcgtgtcattcacaactgctcttaggctactcaggcatggtgagatgctacggtggttgatggatacctagat

SEQ ID NO: 80 - DNA, 34 bp, Artificial Sequence
  Description of Artificial Sequence: Synthetic oligonucleotide
cagaagactcaaagatatctaggtatccatcaac

SEQ ID NO: 81 - DNA, 34 bp, Artificial Sequence
  Description of Artificial Sequence: Synthetic oligonucleotide
gttgatggatacctagatatctttgagtcttctg